European Patent Application EP 4 303 233 A1, published January 10, 2024. Title: TARGETED PROTEIN DEGRADATION SYSTEM AND USE THEREOF. Applicant: ST PHI THERAPEUTICS CO., LTD. The sequence listing filed with the application follows.

SEQUENCE LISTING (178 sequences)

SEQ ID NO: 1 - protein, 144 aa, Homo sapiens
IWSAVFLNSLFNQEVQIPLTESYCGPCPKNWICYKNNCYQFFDESKNWYESQASCMSQNASLLKVYSKEDQDLLKLVKSYHWMGLVHIPTNGSWQWEDGSILSPNLLTIIEMQKGDCALYASSFKGYIENCSTPNTYICMQRTV

SEQ ID NO: 2 - protein, 216 aa, Homo sapiens
MGWIRGRRSRHSWEMSEFHNYNLDLKKSDFSTRWQKQRCPVVKSKCRENASPFFFCCFIAVAMGIRFIIMVTIWSAVFLNSLFNQEVQIPLTESYCGPCPKNWICYKNNCYQFFDESKNWYESQASCMSQNASLLKVYSKEDQDLLKLVKSYHWMGLVHIPTNGSWQWEDGSILSPNLLTIIEMQKGDCALYASSFKGYIENCSTPNTYICMQRTV

SEQ ID NO: 3 - protein, 143 aa, Mus musculus
FKETFQPVLCNKEVPVSSREGYCGPCPNNWICHRNNCYQFFNEEKTWNQSQASCLSQNSSLLKIYSKEEQDFLKLVKSYHWMGLVQIPANGSWQWEDGSSLSYNQLTLVEIPKGSCAVYGSSFKAYTEDCANLNTYICMKRAV

SEQ ID NO: 4 - protein, 232 aa, Mus musculus
MALIRDRKSHHSEMSKCHNYDLKPAKWDTSQEQQKQRLALTTSQPGENGIIRGRYPIEKLKISPMFVVRVLAIALAIRFTLNTLMWLAIFKETFQPVLCNKEVPVSSREGYCGPCPNNWICHRNNCYQFFNEEKTWNQSQASCLSQNSSLLKIYSKEEQDFLKLVKSYHWMGLVQIPANGSWQWEDGSSLSYNQLTLVEIPKGSCAVYGSSFKAYTEDCANLNTYICMKRAV

SEQ ID NO: 5 - protein, 220 aa, Artificial Sequence
MGWIRGRRSRHSWEMSEFHNYNLDLKKSDFSTRWQKQRCPVVKSKCRENASPMFVVRVLAIALAIRFTLNTLMWLAIFKETFQPVLFNQEVQIPLTESYCGPCPKNWICYKNNCYQFFDESKNWYESQASCMSQNASLLKVYSKEDQDLLKLVKSYHWMGLVHIPTNGSWQWEDGSILSPNLLTIIEMQKGDCALYASSFKGYIENCSTPNTYICMQRTV

SEQ ID NO: 6 - protein, 231 aa, Homo sapiens
MSKQRGTFSEVSLAQDPKRQQRKPKGNKSSISGTEQEIFQVELNLQNPSLNHQGIDKIYDCQGLLPPPEKLTAEVLGIICIVLMATVLKTIVLIPFLEQNNSSPNTRTQKARHCGHCPEEWITYSNSCYYIGKERRTWEESLLACTSKNSSLLSIDNEEEMKFLASILPSSWIGVFRNSSHHPWVTINGLAFKHKIKDSDNAELNCAVLQVNRLKSAQCGSSMIYHCKHKL

SEQ ID NO: 7 - protein, 240 aa, Homo sapiens
MSKQRGTFSEVSLAQDPKWQQRKPKGNKSSISGTEQEIFQVELNLQNASLNHQGIDKIYDCQGLLPPPEKLTAEVLGIICIVLMATVLKTIVLIPFLEQNNSSPNARTQKARHCGHCPEEWITYSNSCYYIGKERRTWEESLQACASKNSSSLLCIDNEEEMKFLASILPSSWIGVFRNSSHHPWVTINGLAFKHEIKDSDHAERNCAMLHVRGLISDQCGSSRIIRRGFIMLTRLVLNS

SEQ ID NO: 8 - protein, 158 aa, Homo sapiens
MNKQRGTYSEVSLAQDPKRQQRKLKGNKISISGTKQEIFQVELNLQNASSDHQGNDKTYHCKGLLPPPEKLTAEVLGIICIVLMATVLKTIVLIPCIGVLEQNNFSLNRRMQKARHCGHCPEEWITYSNSCYYIGKERRTWEERVCWPVLRRTLICFL

SEQ ID NO: 9 - protein, 179 aa, Homo sapiens
MAVFKTTLWRLISGTLGIICLSLMSTLGILLKNSFTKLSIEPAFTPGPNIELQKDSDCCSCQEKWVGYRCNCYFISSEQKTWNESRHLCASQKSSLLQLQNTDELDFMSSSQQFYWIGLSYSEEHTAWLWENGSALSQYLFPSFETFNTKNCIAYNPNGNALDESCEDKNRYICKQQLI

SEQ ID NO: 10 - protein, 377 aa, Homo sapiens
MSMSPTVIILACLGFFLDQSVWAHVGGQDKPFCSAWPSAVVPQGGHVTLRCHYRRGFNIFTLYKKDGVPVPELYNRIFWNSFLISPVTPAHAGTYRCRGFHPHSPTEWSAPSNPLVIMVTGLYEKPSLTARPGPTVRAGENVTLSCSSQSSFDIYHLSREGEAHELRLPAVPSINGTFQADFPLGPATHGETYRCFGSFHGSPYEWSDPSDPLPVSVTGNPSSSWPSPTEPSFKTGIARHLHAVIRYSVAIILFTILPFFLLHRWCSKKKDAAVMNQEPAGHRTVNREDSDEQDPQEVTYAQLDHCIFTQRKITGPSQRSKRPSTDTSVCIELPNAEPRALSPAHEHHSQALMGSSRETTALSQTQLASSNVPAAGI

SEQ ID NO: 11 - protein, 304 aa, Homo sapiens
MSLTVVSMACVGFFLLQGAWPHEGVHRKPSLLAHPGRLVKSEETVILQCWSDVMFEHFLLHREGMFNDTLRLIGEHHDGVSKANFSISRMKQDLAGTYRCYGSVTHSPYQLSAPSDPLDIVIIGLYEKPSLSAQPGPTVLAGENVTLSCSSRSSYDMYHLSREGEAHERRLPAGTKVNGTFQANFPLGPATHGGTYRCFGSFRDSPYEWSKSSDPLLVSVTGNPSNSWPSPTEPSSETGNPRHLHVLIGTSVVKIPFTILLFFLLHRWCSDKKNAAVMDQEPAGNRTVNSEDSDEQDHQEVSYA

SEQ ID NO: 12 - protein, 304 aa, Homo sapiens
MSLMVVSMACVGFFLLQGAWPHEGVHRKPSLLAHPGPLVKSEETVILQCWSDVRFEHFLLHREGKYKDTLHLIGEHHDGVSKANFSIGPMMQDLAGTYRCYGSVTHSPYQLSAPSDPLDIVITGLYEKPSLSAQPGPTVLAGESVTLSCSSRSSYDMYHLSREGEAHERRFSAGPKVNGTFQADFPLGPATHGGTYRCFGSFRDSPYEWSNSSDPLLVSVTGNPSNSWPSPTEPSSKTGNPRHLHVLIGTSVVKIPFTILLFFLLHRWCSNKKNAAVMDQEPAGNRTVNSEDSDEQDHQEVSYA

SEQ ID NO: 13 - protein, 304 aa, Homo sapiens
MSLMVIIMACVGFFLLQGAWPQEGVHRKPSFLALPGHLVKSEETVILQCWSDVMFEHFLLHREGKFNNTLHLIGEHHDGVSKANFSIGPMMPVLAGTYRCYGSVPHSPYQLSAPSDPLDMVIIGLYEKPSLSAQPGPTVQAGENVTLSCSSRSSYDMYHLSREGEAHERRLPAVRSINGTFQADFPLGPATHGGTYRCFGSFRDAPYEWSNSSDPLLVSVTGNPSNSWPSPTEPSSKTGNPRHLHVLIGTSVVKIPFTILLFFLLHRWCSDKKNAAVMDQEPAGNRTVNSEDSDEQDHQEVSYA

SEQ ID NO: 14 - protein, 382 aa, Homo sapiens
MLLMVVSMACVGLFLVQRAGPHMGGQDKPFLSAWPSAVVPRGGHVTLRCHYRHRFNNFMLYKEDRIHVPIFHGRIFQEGFNMSPVTTAHAGNYTCRGSHPHSPTGWSAPSNPMVIMVTGNHRKPSLLAHPGPLVKSGERVILQCWSDIMFEHFFLHREWISKDPSRLVGQIHDGVSKANFSIGSMMRALAGTYRCYGSVTHTPYQLSAPSDPLDIVVTGLYEKPSLSAQPGPKVQAGESVTLSCSSRSSYDMYHLSREGGAHERRLPAVRKVNRTFQADFPLGPATHGGTYRCFGSFRHSPYEWSDPSDPLLVSVTGNPSSSWPSPTEPSSKSGNLRHLHILIGTSVVKIPFTILLFFLLHRWCSNKKKCCCNGPRACREQK

SEQ ID NO: 15 - protein, 304 aa, Homo sapiens
MSSTLPALLCVGLCLSQRISAQQQTLPKPFIWAEPHFMVPKEKQVTICCQGNYGAVEYQLHFEGSLFAVDRPKPPERINKVKFYIPDMNSRMAGQYSCIYRVGELWSEPSNLLDLVVTEMYDTPTLSVHPGPEVISGEKVTFYCRLDTATSMFLLLKEGRSSHVQRGYGKVQAEFPLGPVTTAHRGTYRCFGSYNNHAWSFPSEPVKLLVTGDIENTSLAPEDPTFPADTWGTYLLTTETGLQKDHALWDHTAQNLLRMGLAFLVLVALVWFLVEDWLSRKRTRERASRASTWEGRRRLNTQTL

SEQ ID NO: 16 - protein, 276 aa, Homo sapiens
MAWRALHPLLLLLLLFPGSQAQSKAQVLQSVAGQTLTVRCQYPPTGSLYEKKGWCKEASALVCIRLVTSSKPRTMAWTSRFTIWDDPDAGFFTVTMTDLREEDSGHYWCRIYRPSDNSVSKSVRFYLVVSPASASTQTSWTPRDLVSSQTQTQSCVPPTAGARQAPESPSTIPVPSQPQNSTLRPGPAAPIALVPVFCGLLVAKSLVLSALLVWWGDIWWKTMMELRSLDTQKATCHLQQVTDLPWTSVSSPVEREILYHTVARTKISDDDDEHTL

SEQ ID NO: 17 - protein, 201 aa, Homo sapiens
MAWMLLLILIMVHPGSCALWVSQPPEIRTLEGSSAFLPCSFNASQGRLAIGSVTWFRDEVVPGKEVRNGTPEFRGRLAPLASSRFLHDHQAELHIRDVRGHDASIYVCRVEVLGLGVGTGNGTRLVVEKEHPQLGAGTVLLLRAGFYAVSFLSVAVGSTVYYQGKCLTWKGPRRQLPAVVPAPLPPPCGSSAHLLPPVPGG

SEQ ID NO: 18 - protein, 336 aa, Homo sapiens
MDYPTLLLALLHVYRALCEEVLWHTSVPFAENMSLECVYPSMGILTQVEWFKIGTQQDSIAIFSPTHGMVIRKPYAERVYFLNSTMASNNMTLFFRNASEDDVGYYSCSLYTYPQGTWQKVIQVVQSDSFEAAVPSNSHIVSEPGKNVTLTCQPQMTWPVQAVRWEKIQPRQIDLLTYCNLVHGRNFTSKFPRQIVSNCSHGRWSVIVIPDVTVSDSGLYRCYLQASAGENETFVMRLTVAEGKTDNQYTLFVAGGTVLLLLFVISITTIIVIFLNRRRRRERRDLFTESWDTQKAPNNYRSPISTSQPTNQSMDDTREDIYVNYPTFSRRPKTRV

SEQ ID NO: 19 - protein, 281 aa, Homo sapiens [sequence omitted]

SEQ ID NO: 20 - protein, 254 aa, Homo sapiens
MWQLLLPTALLLLVSAGMRTEDLPKAVVFLEPQWYRVLEKDSVTLKCQGAYSPEDNSTQWFHNESLISSQASSYFIDAATVDDSGEYRCQTNLSTLSDPVQLEVHIGWLLLQAPRWVFKEEDPIHLRCHSWKNTALHKVTYLQNGKGRKYFHHNSDFYIPKATLKDSGSYFCRGLFGSKNVSSETVNITITQGLAVSTISSFFPPGYQVSFCLVMVLLFAVDTGLYFSVKTNIRSSTRDWKDHKFKWRKDPQDK

SEQ ID NO: 21 - protein, 370 aa, Homo sapiens
MLGQVVTLILLLLLKVYQGKGCQGSADHVVSISGVPLQLQPNSIQTKVDSIAWKKLLPSQNGFHHILKWENGSLPSNTSNDRFSFIVKNLSLLIKAAQQQDSGLYCLEVTSISGKVQTATFQVFVFESLLPDKVEKPRLQGQGKILDRGRCQVALSCLVSRDGNVSYAWYRGSKLIQTAGNLTYLDEEVDINGTHTYTCNVSNPVSWESHTLNLTQDCQNAHQEFRFWPFLVIIVILSALFLGTLACFCVWRRKRKEKQSETSPKEFLTIYEDVKDLKTRRNHEQEQTFPGGGSTIYSMIQSQSSAPTSQEPAYTLYSLIQPSRKSGSRKRNHSPSFNSTIYEVIGKSQPKAQNPARLSRKELENFDVYS

SEQ ID NO: 22 - protein, 332 aa, Homo sapiens
MLWLFQSLLFVFCFGPGNVVSQSSLTPLMVNGILGESVTLPLEFPAGEKVNFITWLFNETSLAFIVPHETKSPEIHVTNPKQGKRLNFTQSYSLQLSNLKMEDTGSYRAQISTKTSAKLSSYTLRILRQLRNIQVTNHSQLFQNMTCELHLTCSVEDADDNVSFRWEALGNTLSSQPNLTVSWDPRISSEQDYTCIAENAVSNLSFSVSAQKLCEDVKIQYTDTKMILFMVSGICIVFGFIILLLLVLRKRRDSLSLSTQRTQGPAESARNLEYVSVSPTNNTVYASVTHSNRETEIWTPRENDTITIYSTINHSKESKPTFSRATALDNVV

SEQ ID NO: 23 - protein, 335 aa, Homo sapiens
MAGSPTCLTLIYILWQLTGSAASGPVKELVGSVGGAVTFPLKSKVKQVDSIVWTFNTTPLVTIQPEGGTIIVTQNRNRERVDFPDGGYSLKLSKLKKNDSGIYYVGIYSSSLQQPSTQEYVLHVYEHLSKPKVTMGLQSNKNGTCVTNLTCCMEHGEEDVIYTWKALGQAANESHNGSILPISWRWGESDMTFICVARNPVSRNFSSPILARKLCEGAADDPDSSMVLLCLLLVPLLLSLFVLGLFLWFLKRERQEEYIEEKKRVDICRETPNICPHSGENTEYDTIPHTNRTILKEDPANTVYSTVEIPKKMENPHSLLTMPDTPRLFAYENVI

SEQ ID NO: 24 - protein, 231 aa, Homo sapiens
MQDEERYMTLNVQSKKRSSAQTSQLTFKDYSVTLHWYKILLGISGTVNGILTLTLISLILLVSQGVLLKCQKGSCSNATQYEDTGDLKVNNGTRRNISNKDLCASRSADQTVLCQSEWLKYQGKCYWFSNEMKSWSDSYVYCLERKSHLLIIHDQLEMAFIQKNLRQLNYVWIGLNFTSLKMTWTWVDGSPIDSKIFFIKGPAKENSCAAIKESKIFSETCSSVFKWICQY

SEQ ID NO: 25 - protein, 93 aa, Homo sapiens
MIHLGHILFLLLLPVAAAQTTPGERSSLPAFYPGTSGSCSGCGSLSLPLLAGLVAADAVASLLIVGAVFLCARPRRSPAQEDGKVYINMPGRG

SEQ ID NO: 26 - protein, 92 aa, Homo sapiens
MIHLGHILFLLLLPVAAAQTTPGERSSLPAFYPGTSGSCSGCGSLSLPLLAGLVAADAVASLLIVGAVFLCARPRRSPAQDGKVYINMPGRG

SEQ ID NO: 27 - protein, 21 aa, Homo sapiens
LLAGLVAADAVASLLIVGAVF

SEQ ID NO: 28 - protein, 113 aa, Homo sapiens
MGGLEPCSRLLLLPLLLAVSGLRPVQAQAQSDCSCSTVSPGVLAGIVMGDLVLTVLIALAVYFLGRLVPRGRGAAEAATRKQRITETESPYQELQGQRSDVYSDLNTQRPYYK

SEQ ID NO: 29 - protein, 21 aa, Homo sapiens
GVLAGIVMGDLVLTVLIALAV

SEQ ID NO: 30 - protein, 38 aa, Artificial Sequence
GVLAGIVMGDLVLTVLIALAVLVAADAVASLLIVGAVF

SEQ ID NO: 31 - protein, 150 aa, Artificial Sequence
MIHLGHILFLLLLPVAAAQTTPGERSSLPAFYPGTSGSCSGCGSLSLPLLAGLVAADAVASLLIVGAVFLCARPRRSPAQEDGKVYINMPGRGGGGGSYFLGRLVPRGRGAAEAATRKQRITETESPYQELQGQRSDVYSDLNTQRPYYK

SEQ ID NO: 32 - protein, 112 aa, Homo sapiens
RVKFSRSADAPAYQQGQNQLYNELNLGRREEYDVLDKRRGRDPEMGGKPRRKNPQEGLYNELQKDKMAEAYSEIGMKGERRRGKGHDGLYQGLSTATKDTYDALHMQALPPR

SEQ ID NO: 33 - protein, 210 aa, Artificial Sequence
MIHLGHILFLLLLPVAAAQTTPGERSSLPAFYPGTSGSCSGCGSLSLPLLAGLVAADAVASLLIVGAVFLCARPRRSPAQEDGKVYINMPGRGGGGGSRVKFSRSADAPAYQQGQNQLYNELNLGRREEYDVLDKRRGRDPEMGGKPRRKNPQEGLYNELQKDKMAEAYSEIGMKGERRRGKGHDGLYQGLSTATKDTYDALHMQALPPR

SEQ ID NO: 34 - protein, 230 aa, Artificial Sequence
MGGLEPCSRLLLLPLLLAVSGLRPVQAQAQSDCSCSTVSPGVLAGIVMGDLVLTVLIALAVYFLGRLVPRGRGAAEAATRKQRITETESPYQELQGQRSDVYSDLNTQRPYYKGGGGSRVKFSRSADAPAYQQGQNQLYNELNLGRREEYDVLDKRRGRDPEMGGKPRRKNPQEGLYNELQKDKMAEAYSEIGMKGERRRGKGHDGLYQGLSTATKDTYDALHMQALPPR

SEQ ID NO: 35 - protein, 267 aa, Artificial Sequence
MIHLGHILFLLLLPVAAAQTTPGERSSLPAFYPGTSGSCSGCGSLSLPLLAGLVAADAVASLLIVGAVFLCARPRRSPAQEDGKVYINMPGRGGGGGSYFLGRLVPRGRGAAEAATRKQRITETESPYQELQGQRSDVYSDLNTQRPYYKGGGGSRVKFSRSADAPAYQQGQNQLYNELNLGRREEYDVLDKRRGRDPEMGGKPRRKNPQEGLYNELQKDKMAEAYSEIGMKGERRRGKGHDGLYQGLSTATKDTYDALHMQALPPR

SEQ ID NO: 36 - protein, 42 aa, Homo sapiens
KRGRKKLLYIFKQPFMRPVQTTQEEDGCSCRFPEEEEGGCEL

SEQ ID NO: 37 - protein, 140 aa, Artificial Sequence
MIHLGHILFLLLLPVAAAQTTPGERSSLPAFYPGTSGSCSGCGSLSLPLLAGLVAADAVASLLIVGAVFLCARPRRSPAQEDGKVYINMPGRGGGGGSKRGRKKLLYIFKQPFMRPVQTTQEEDGCSCRFPEEEEGGCEL

SEQ ID NO: 38 - protein, 252 aa, Artificial Sequence
MIHLGHILFLLLLPVAAAQTTPGERSSLPAFYPGTSGSCSGCGSLSLPLLAGLVAADAVASLLIVGAVFLCARPRRSPAQEDGKVYINMPGRGGGGGSKRGRKKLLYIFKQPFMRPVQTTQEEDGCSCRFPEEEEGGCELRVKFSRSADAPAYQQGQNQLYNELNLGRREEYDVLDKRRGRDPEMGGKPRRKNPQEGLYNELQKDKMAEAYSEIGMKGERRRGKGHDGLYQGLSTATKDTYDALHMQALPPR

SEQ ID NO: 39 - protein, 41 aa, Homo sapiens
RSKRSRLLHSDYMNMTPRRPGPTRKHYQPYAPPRDFAAYRS

SEQ ID NO: 40 - protein, 139 aa, Artificial Sequence
MIHLGHILFLLLLPVAAAQTTPGERSSLPAFYPGTSGSCSGCGSLSLPLLAGLVAADAVASLLIVGAVFLCARPRRSPAQEDGKVYINMPGRGGGGGSRSKRSRLLHSDYMNMTPRRPGPTRKHYQPYAPPRDFAAYRS

SEQ ID NO: 41 - protein, 251 aa, Artificial Sequence
MIHLGHILFLLLLPVAAAQTTPGERSSLPAFYPGTSGSCSGCGSLSLPLLAGLVAADAVASLLIVGAVFLCARPRRSPAQEDGKVYINMPGRGGGGGSRSKRSRLLHSDYMNMTPRRPGPTRKHYQPYAPPRDFAAYRSRVKFSRSADAPAYQQGQNQLYNELNLGRREEYDVLDKRRGRDPEMGGKPRRKNPQEGLYNELQKDKMAEAYSEIGMKGERRRGKGHDGLYQGLSTATKDTYDALHMQALPPR

SEQ ID NO: 42 - protein, 160 aa, Artificial Sequence
MGGLEPCSRLLLLPLLLAVSGLRPVQAQAQSDCSCSTVSPGVLAGIVMGDLVLTVLIALAVYFLGRLVPRGRGAAEAATRKQRITETESPYQELQGQRSDVYSDLNTQRPYYKGGGGSKRGRKKLLYIFKQPFMRPVQTTQEEDGCSCRFPEEEEGGCEL

SEQ ID NO: 43 - protein, 272 aa, Artificial Sequence
MGGLEPCSRLLLLPLLLAVSGLRPVQAQAQSDCSCSTVSPGVLAGIVMGDLVLTVLIALAVYFLGRLVPRGRGAAEAATRKQRITETESPYQELQGQRSDVYSDLNTQRPYYKGGGGSKRGRKKLLYIFKQPFMRPVQTTQEEDGCSCRFPEEEEGGCELRVKFSRSADAPAYQQGQNQLYNELNLGRREEYDVLDKRRGRDPEMGGKPRRKNPQEGLYNELQKDKMAEAYSEIGMKGERRRGKGHDGLYQGLSTATKDTYDALHMQALPPR

SEQ ID NO: 44 - protein, 159 aa, Artificial Sequence
MGGLEPCSRLLLLPLLLAVSGLRPVQAQAQSDCSCSTVSPGVLAGIVMGDLVLTVLIALAVYFLGRLVPRGRGAAEAATRKQRITETESPYQELQGQRSDVYSDLNTQRPYYKGGGGSRSKRSRLLHSDYMNMTPRRPGPTRKHYQPYAPPRDFAAYRS

SEQ ID NO: 45 - protein, 271 aa, Artificial Sequence
MGGLEPCSRLLLLPLLLAVSGLRPVQAQAQSDCSCSTVSPGVLAGIVMGDLVLTVLIALAVYFLGRLVPRGRGAAEAATRKQRITETESPYQELQGQRSDVYSDLNTQRPYYKGGGGSRSKRSRLLHSDYMNMTPRRPGPTRKHYQPYAPPRDFAAYRSRVKFSRSADAPAYQQGQNQLYNELNLGRREEYDVLDKRRGRDPEMGGKPRRKNPQEGLYNELQKDKMAEAYSEIGMKGERRRGKGHDGLYQGLSTATKDTYDALHMQALPPR

SEQ ID NO: 46 - protein, 199 aa, Human cytomegalovirus
MNNLWKAWVGLWTSMGPLIRLPDGITKAGEDALRPWKSTAKHPWFEIEDNRCYIDNGKLFARGSIVGNMSRFVFDPKADYGGVGENLYVHADDVEFVPGESLKWNVRNLDVMPIFETLALRLVLQGDVIWLRCVPELRVDYTSSAYMWNMQYGMVRKSYTHVAWTIVFYSINITLLVLFIVYVTVDCNLSMMWMRFFVC

SEQ ID NO: 47 - protein, 161 aa, Human cytomegalovirus
MNNLWKAWVGLWTSMGPLIRLPDGITKAGEDALRPWKSTAKHPWFEIEDNRCYIDNGKLFARGSIVGNMSRFVFDPKADYGGVGENLYVHADDVEFVPGESLKWNVRNLDVMPIFETLALRLVLQGDVIWLRCVPELRVDYTSSAYMWNMQYGMVRKSYTH

SEQ ID NO: 48 - protein, 38 aa, Human cytomegalovirus
VAWTIVFYSINITLLVLFIVYVTVDCNLSMMWMRFFVC

SEQ ID NO: 49 - protein, 186 aa, Human cytomegalovirus
MKPVLVLAILAVLFLRLADSVPRPLDVVVSEIRSAHFRVEENQCWFHMGMLYFKGRMSGNFTEKHFVNVGIVSQSYMDRLQVSGEQYHHDERGAYFEWNIGGHPVTHTVDMVDITLSTRWGDPKKYAACVPQVRMDYSSQTINWYLQRSMRDDNWGLLFRTLLVYLFSLVVLVLLTVGVSARLRFI

SEQ ID NO: 50 - protein, 160 aa, Human cytomegalovirus
MKPVLVLAILAVLFLRLADSVPRPLDVVVSEIRSAHFRVEENQCWFHMGMLYFKGRMSGNFTEKHFVNVGIVSQSYMDRLQVSGEQYHHDERGAYFEWNIGGHPVTHTVDMVDITLSTRWGDPKKYAACVPQVRMDYSSQTINWYLQRSMRDDNWGLLFR

SEQ ID NO: 51 - protein, 26 aa, Human cytomegalovirus
TLLVYLFSLVVLVLLTVGVSARLRFI

SEQ ID NO: 52 - protein, 215 aa, Human cytomegalovirus
MNLVMLILALWAPVAGSMPELSLTLFDEPPPLVETEPLPPLSDVSEYRVEYSEARCVLRSGGRLEALWTLRGNLSVPTPTPRVYYQTLEGYADRVPTPVEDVSESLVAKRYWLRDYRVPQRTKLVLFYFSPCHQCQTYYVECEPRCLVPWVPLWSSLEDIERLLFEDRRLMAYYALTIKSAQYTLMMVAVIQVFWGLYVKGWLHRHFPWMFSDQW

SEQ ID NO: 53 - protein, 165 aa, Human cytomegalovirus
MPELSLTLFDEPPPLVETEPLPPLSDVSEYRVEYSEARCVLRSGGRLEALWTLRGNLSVPTPTPRVYYQTLEGYADRVPTPVEDVSESLVAKRYWLRDYRVPQRTKLVLFYFSPCHQCQTYYVECEPRCLVPWVPLWSSLEDIERLLFEDRRLMAYYALTIKSAQ

SEQ ID NO: 54 - protein, 33 aa, Human cytomegalovirus
YTLMMVAVIQVFWGLYVKGWLHRHFPWMFSDQW

SEQ ID NO: 55 - protein, 185 aa, Human cytomegalovirus
MLRRGSLRNPLAICLLWWLGVVAAATEETREPTYFTCGCVIQNHVLKGAVKLYGQFPSPKTLRASAWLHDGENHERHRQPILVEGTATATEALYILLPTELSSPEGNRPRNYSATLTLASRDCYERFVCPVYDSGTPMGVLMNLTYLWYLGDYGAILKIYFGLFCGACVITRSLLLICGYYPPRE

SEQ ID NO: 56 - protein, 124 aa, Human cytomegalovirus
ATEETREPTYFTCGCVIQNHVLKGAVKLYGQFPSPKTLRASAWLHDGENHERHRQPILVEGTATATEALYILLPTELSSPEGNRPRNYSATLTLASRDCYERFVCPVYDSGTPMGVLMNLTYLW

SEQ ID NO: 57 - protein, 36 aa, Human cytomegalovirus
LGDYGAILKIYFGLFCGACVITRSLLLICGYYPPRE

SEQ ID NO: 58 - protein, 159 aa, Adenovirus type 37
MRYMILGLLALAAVCSAAKKVEFKEPACNVTFKSEANECTTLIKCTTEHEKLIIRHKDKIGKYAVYAIWQPGDTNDYNVTVFQGENRKTFMYKFPFYEMCDITMYMSKQYKLWPPQKCLENTGTFCSTALLITALALVCTLLYLKYKSRRSFIDEKKMP

SEQ ID NO: 59 - protein, 106 aa, Adenovirus type 37
AKKVEFKEPACNVTFKSEANECTTLIKCTTEHEKLIIRHKDKIGKYAVYAIWQPGDTNDYNVTVFQGENRKTFMYKFPFYEMCDITMYMSKQYKLWPPQKCLENTG

SEQ ID NO: 60 - protein, 36 aa, Adenovirus type 37
TFCSTALLITALALVCTLLYLKYKSRRSFIDEKKMP

SEQ ID NO: 61 - protein, 430 aa, human herpesvirus 1
MWTILLFCVPVIYGELYPDFCPLAVVDFDVNATVDDLLLFDISLSKQCSDDKIRHSAVAAMTDNAFFFGNSETQIETDFGKYLAFNCYQVFSTLNHFLFKNFKKTKGLMKRYDKLCLDVESYIHIQIICSPFKSFIRLRRMNETGISPRILETTFYLQNKRNSTWVAIKNYLGEDDPFTYRIWHTLTHAKNFLINSCENDFNQLFFWQRKYLSLAKTFEATFKQGFNPMIEQRNEQRYRTNNIDCSFSKFRQNGVKVAVCKYTGWGVSGFGSLEVLQKIKSPFGEEWKRVGFNSTGAFTPLYGSDVLWGLIFLRVEMTTYVCTCTNKNTGTQIQVTLPDVDLDLLDSEKTSSNVFVDMLCYTLIAILFLAFVTAVVLLGVSCLDGVQKVLTWPLQHIQKEPVSEKIINLTNLMFGQEPLPKKESLKQQCL

SEQ ID NO: 62 - protein, 362 aa, human herpesvirus 1
MWTILLFCVPVIYGELYPDFCPLAVVDFDVNATVDDLLLFDISLSKQCSDDKIRHSAVAAMTDNAFFFGNSETQIETDFGKYLAFNCYQVFSTLNHFLFKNFKKTKGLMKRYDKLCLDVESYIHIQIICSPFKSFIRLRRMNETGISPRILETTFYLQNKRNSTWVAIKNYLGEDDPFTYRIWHTLTHAKNFLINSCENDFNQLFFWQRKYLSLAKTFEATFKQGFNPMIEQRNEQRYRTNNIDCSFSKFRQNGVKVAVCKYTGWGVSGFGSLEVLQKIKSPFGEEWKRVGFNSTGAFTPLYGSDVLWGLIFLRVEMTTYVCTCTNKNTGTQIQVTLPDVDLDLLDSEKTSSNVFVDMLCYT

SEQ ID NO: 63 - protein, 68 aa, human herpesvirus 1
LIAILFLAFVTAVVLLGVSCLDGVQKVLTWPLQHIQKEPVSEKIINLTNLMFGQEPLPKKESLKQQCL

SEQ ID NO: 64 - protein, 183 aa, Human cytomegalovirus
MDLLIRLGFLLMCALPTPGERSSRDPKTLLSLSPRQQACVPRTKSHRPVCYNDTGDCTDADDSWKQLGEDFAHQCLQAAKKRPKTHKSRPNDRNLEGRLTCQRVRRLLPCDLDIHPSHRLLTLMNNCVCDGAVWNAFRLIERHGFFAVTLYLCCGITLLVVILALLCSITYESTGRGIRRCGS

SEQ ID NO: 65 - protein, 125 aa, Human cytomegalovirus
ERSSRDPKTLLSLSPRQQACVPRTKSHRPVCYNDTGDCTDADDSWKQLGEDFAHQCLQAAKKRPKTHKSRPNDRNLEGRLTCQRVRRLLPCDLDIHPSHRLLTLMNNCVCDGAVWNAFRLIERHG

SEQ ID NO: 66 - protein, 88 aa, herpes simplex virus 7
MSWALEMADTFLDTMRVGPRTYADVRDEINKRGREDREAARTAVHDPERPLLRSPGLLPEIAPNASLGVAHRRTGGTVTDSPRNPVTR

SEQ ID NO: 67 - protein, 57 aa, herpes simplex virus 7
MSWALEMADTFLDTMRVGPRTYADVRDEINKRGREDREAARTAVHDPERPLLRSPGL

SEQ ID NO: 68 - protein, 160 aa, Cowpox virus
MFIMRELVYRVVIVILSLSLLSSFLVICFIEHRCFKEETRYKICPKNTISINNICYYFSEDTTNWTASFEYCKNMNGRLACIINDTFPKICRYKGTFDYWVGLYRTNSQSPWLNCDNKPYNNIIPIRGVEDYAYLNNNGISTARIYADRRWICEVPMVDY

SEQ ID NO: 69 - protein, 133 aa, Cowpox virus
CFIEHRCFKEETRYKICPKNTISINNICYYFSEDTTNWTASFEYCKNMNGRLACIINDTFPKICRYKGTFDYWVGLYRTNSQSPWLNCDNKPYNNIIPIRGVEDYAYLNNNGISTARIYADRRWICEVPMVDY

SEQ ID NO: 70 - protein, 60 aa, Epstein Barr virus
MVHVLERALLEQQSSACGLPGSSTETRPSHPCPEDPDVSRLRLLLAVLCVLFGLLCLLLI

SEQ ID NO: 71 - protein, 40 aa, Epstein Barr virus
MVHVLERALLEQQSSACGLPGSSTETRPSHPCPEDPDVSR

SEQ ID NO: 72 - protein, 96 aa, Bovine herpesvirus 1
MPRSPLIVAVVAAALFAIVRGRDPLLDAMRREGAMDFWSAGCYARGVPLSEPPQALVVFYVALTAVMVAVALYAYGLCFRLMGASGPNKKESRGRG

SEQ ID NO: 73 - protein, 54 aa, Bovine herpesvirus 1
MPRSPLIVAVVAAALFAIVRGRDPLLDAMRREGAMDFWSAGCYARGVPLSEPPQ

SEQ ID NO: 74 - protein, 199 aa, Human cytomegalovirus; identical to SEQ ID NO: 46

SEQ ID NO: 75 - protein, 161 aa, Human cytomegalovirus; identical to SEQ ID NO: 47

SEQ ID NO: 76 - protein, 38 aa, Human cytomegalovirus; identical to SEQ ID NO: 48

SEQ ID NO: 77 - protein, 186 aa, Human cytomegalovirus; identical to SEQ ID NO: 49

SEQ ID NO: 78 - protein, 160 aa, Human cytomegalovirus; identical to SEQ ID NO: 50

SEQ ID NO: 79 - protein, 26 aa, Human cytomegalovirus
TLLVYLFSLVVLVLLTVGVSARLRFI

SEQ ID NO: 80 - protein, 215 aa, Human cytomegalovirus; identical to SEQ ID NO: 52

SEQ ID NO: 81 - protein, 165 aa, Human cytomegalovirus; identical to SEQ ID NO: 53

SEQ ID NO: 82 - protein, 33 aa, Human cytomegalovirus; identical to SEQ ID NO: 54

SEQ ID NO: 83 - protein, 230 aa, Human cytomegalovirus
MERRRGTVPLGWVFFVLCLSASSSCAVDLGSKSSNSTCRLNVTELASIHPGETWTLHGMCISICYYENVTEDEIIGVAFTWQHNESVVDLWLYQNDTVIRNFSDITTNILQDGLKMRTVPVTKLYTSRMVTNLTVGRYDCLRCENGTTKIIERLYVRLGSLYPRPPGSGLAKHPSVSADEELSATLARDIVLVSAITLFFFLLALRIPQRLCQRLRIRLPHRYQRLRTED

SEQ ID NO: 84 - protein, 158 aa, Human cytomegalovirus
VDLGSKSSNSTCRLNVTELASIHPGETWTLHGMCISICYYENVTEDEIIGVAFTWQHNESVVDLWLYQNDTVIRNFSDITTNILQDGLKMRTVPVTKLYTSRMVTNLTVGRYDCLRCENGTTKIIERLYVRLGSLYPRPPGSGLAKHPSVSADEELSA

SEQ ID NO: 85 - protein, 46 aa, Human cytomegalovirus
TLARDIVLVSAITLFFFLLALRIPQRLCQRLRIRLPHRYQRLRTED

SEQ ID NO: 86 - protein, 338 aa, Human cytomegalovirus
MCRRESLRTLPWLFWVLLSCPRLLEYSSSSFPFATADIAEKMWAENYETTSPAPVLVAEGEQVTIPCTVMTHSWPMVSIRARFCRSHDGSDELILDAVKGHRLMNGLQYRLPYATWNFSQLHLGQIFSLTFNVSTDTAGMYECVLRNYSHGLIMQRFVILTQLETLSRPDEPCCTPALGRYSLGDQIWSPTPWRLRNHDCGMYRGFQRNYFYIGRADAEDCWKPACPDEEPDRCWTVIQRYRLPGDCYRSQPHPPKFLPVTPAPPADIDTGMSPWATRGIAAFLGFWSIFTVCFLCYLCYLQCCGRWCPTPGRGRRGGEGYRRLPTYDSYPGVKKMKR

SEQ ID NO: 87 - protein, 242 aa, Human cytomegalovirus
DIAEKMWAENYETTSPAPVLVAEGEQVTIPCTVMTHSWPMVSIRARFCRSHDGSDELILDAVKGHRLMNGLQYRLPYATWNFSQLHLGQIFSLTFNVSTDTAGMYECVLRNYSHGLIMQRFVILTQLETLSRPDEPCCTPALGRYSLGDQIWSPTPWRLRNHDCGMYRGFQRNYFYIGRADAEDCWKPACPDEEPDRCWTVIQRYRLPGDCYRSQPHPPKFLPVTPAPPADIDTGMSPWATR

SEQ ID NO: 88 - protein, 60 aa, Human cytomegalovirus
GIAAFLGFWSIFTVCFLCYLCYLQCCGRWCPTPGRGRRGGEGYRRLPTYDSYPGVKKMKR

SEQ ID NO: 89 - protein, 305 aa, Human cytomegalovirus
MRIEWACWLFGYFVSSVGSERSLSYRYHLESNSSANVVCNGNISVFVNGTLGVRYNITVGISSSLLIGHLTIQTLESWFTPWVQNKSYSKQPLSTTETLYNIDSENIHRVSQYFHTRWIKSLQENHTCDLTNSTPTYTYQANVNNTNYLTLTSSGWQDRLNYTAINSTHFNLTESNITSIHKYLNTTCIERLRNYTLEPVYTTAVPQNVTPEHAITTLYTTPPNAITIKDTTQSHTVQTPSFNDTHNVTEHTLNISYVLSQKTNNTTSPWVYAIPMGATATIGAGLYIGKHFTPVKFVYEVWRGQ

SEQ ID NO: 90 - protein, 251 aa, Human cytomegalovirus
ERSLSYRYHLESNSSANVVCNGNISVFVNGTLGVRYNITVGISSSLLIGHLTIQTLESWFTPWVQNKSYSKQPLSTTETLYNIDSENIHRVSQYFHTRWIKSLQENHTCDLTNSTPTYTYQANVNNTNYLTLTSSGWQDRLNYTAINSTHFNLTESNITSIHKYLNTTCIERLRNYTLEPVYTTAVPQNVTPEHAITTLYTTPPNAITIKDTTQSHTVQTPSFNDTHNVTEHTLNISYVLSQKTNNTTSPW

SEQ ID NO: 91 - protein, 35 aa, Human cytomegalovirus
VYAIPMGATATIGAGLYIGKHFTPVKFVYEVWRGQ

SEQ ID NO: 92 - protein, 205 aa, Human immunodeficiency virus
MGGKWSKSKTAGWPEVRERIRNAPSAAAPGVGAVSQDLAKHGAITSSNANHPSCVWLEAQEDEEVGFPVRPQVPLRPMTYKGALDLSHFLKEKGGLEGLIYSRRRQEILDLWVYHTQGYFPDWQNYTPGPGIRYPLTFGWCFKLVPVEPEEVEKATEGENNSLLHPICQHGMDDEEGEVLKWQFDPRLALKHRAQELHPEFYKDC

SEQ ID NO: 93 - protein, 81 aa, Human immunodeficiency virus
QPIPIVAIVALVVAIIIAIVVWSIVIIEYRKILRQRKIDRLIDRLIERAEDSGNESEGEISALVEMGVEMGHHAPWDVDDL

SEQ ID NO: 94 - protein, 333 aa, Human herpesvirus type 4
MEDEDVPVCWICNEELGNERFRACGCTGELENVHRSCLSTWLTISRNTACQICGVVYNTRVVWRPLREMTLLPRLTYQEGLELIVFIFIMTLGAAGLAAATWVWLYIVGGHDPEIDHVAAAAYYVFFVFYQLFVVFGLGAFFHMMRHVGRAYAAVNTRVEVFPYRPRPTSPECAVEEIELQEILPRGDNQDEEGPAGAAPGDQNGPAGAAPGDQDGPADGAPVHRDSEESVDEAAGYKEAGEPTHNDGRDDNVEPTAVGCDCNNLGAERYRATYCGGYVGAQSGDGAYSVSCHNKAGPSSLVDILPQGLPGGGYGSMGVIRKRSAVSSALMFH

SEQ ID NO: 95 - protein, 256 aa, Human herpesvirus type 4
MASKDVEEGVEGPICWICREEVGNEGIHPCACTGELDVVHPQCLSTWLTVSRNTACQMCRVIYRTRTQWRSRLNLWPEMERQEIFELFLLMSVVVAGLVGVALCTWTLLVILTAPAGTFSPGAVLGFLCFFGFYQIFIVFAFGGICRVSGTVRALYAANNTRVTVLPYRRPRRPTANEDNIELTVLVGPAGGTDEEPTDESSEGDVASGDKERDGSSGDEPDGGPNDRAGLRGTARTDLCAPTKKPVRKNHPKNNG

SEQ ID NO: 96 - protein, 201 aa, Human herpesvirus type 4
MDSTGEFCWICHQPEGPLKRFCGCKGSCAVSHQDCLRGWLETSRRQTCALCGTPYSMKWKTKPLREWTWGEEEVLAAMEACLPLVLIPLAVLMIVMGTWLLVNHNGFLSPRMQVVLVVIVLLAMIVFSASASYVMVEGPGCLDTCTAKNSTVTVNSIDEAIATQQPTKTDLGLARETLSTRFRRGKCRSCCRLGCVRLCCV

SEQ ID NO: 97 - protein, 99 aa, Human T-cell lymphotropic virus
MLFRLLSPLSPLALTALLLFLLPPSDVSGLLLRPPPAPCLLLFLPFQILSGLLFLLFLPLFFSLPLLLSPSLPITMRFPARWRFLPWKAPSQPAAAFLF

SEQ ID NO: 98 - protein, 245 aa, Cowpox virus
MKIKLSIIRWLTLLALTIFRMRSLVIVLLFPSIIYSMVIRRCEKMEEETWKLKIGMCIQAKDFYSKRTDCSVHRSDVGGGLITEGNGYRVVVHDQCEEPNPFIIATTKQTHFGVTHSYIEFSNSNTGAPENIPDCSKHILISVYCDQEASGLDFHTLKYVESNYLHITVKYDTSCINHLGVNYSFMNECERKLKSIYETDTLTCGAKDTQTRDKYLKTCTNTKFDRSVYKTHMQKSKILHVKTEL

SEQ ID NO: 99 - protein, 234 aa, Cowpox virus
MKIKLSIIRWLTLLALTIFRMRSLVIVLLFPSIIYSMVIRRCEKMEEETWKLKIGMCIQAKDFYSKRTDCSVHRSDVGGGLITEGNGYRVVVHDQCEEPNPFIIATTKQTHFGVTHSYIEFSNSNTGAPENIPDCSKHILISVYCDQEASGLDFHTLKYVESNYLHITVKYDTSCINHLGVNYSFMNECERKLKSIYETDTLTCGAKDTQTRDKYLKTCTNTKFDRSVYKTHMQ

SEQ ID NO: 100 - protein, 11 aa, Cowpox virus
KSKILHVKTEL

SEQ ID NO: 101 - protein, 245 aa, Cowpox virus
MKIKLSIIRWLTLLALTIFRMRSLIIFLLFPSIIYSMVIRRCEKMEEETWKLKIGMCIQAKDFYSKRTDCSVHRSDVGGGLITEGNGYRVVVHDQCEEPNPFIIATTKQTHFGVTHSYIEFSNSNTGAPENIPDCSKHILISVYCDQEASGLDFHTLKYVESNYLHITVKYDTSCINHLGVNYSFMNECERKLKSIYETDTLTCGAKDTQTRDKYLKTCTNTKFDRSVYKTHMRKSKILHVKTEL

SEQ ID NO: 102 - protein, 234 aa, Cowpox virus
MKIKLSIIRWLTLLALTIFRMRSLIIFLLFPSIIYSMVIRRCEKMEEETWKLKIGMCIQAKDFYSKRTDCSVHRSDVGGGLITEGNGYRVVVHDQCEEPNPFIIATTKQTHFGVTHSYIEFSNSNTGAPENIPDCSKHILISVYCDQEASGLDFHTLKYVESNYLHITVKYDTSCINHLGVNYSFMNECERKLKSIYETDTLTCGAKDTQTRDKYLKTCTNTKFDRSVYKTHMR

SEQ ID NO: 103 - protein, 11 aa, Cowpox virus
KSKILHVKTEL

SEQ ID NO: 104 - protein, 5 aa, Artificial Sequence
GGGGS

SEQ ID NO: 105 - protein, 8 aa, Artificial Sequence
GGGSGGGS

SEQ ID NO: 106 - protein, 15 aa, Homo sapiens
EPKSCDKTHTCPPCP

SEQ ID NO: 107 - protein, 12 aa, Homo sapiens
ESKYGPPCPSCP

SEQ ID NO: 108 - protein, 18 aa, Homo sapiens
EGRGSLLTCGDVEENPGP

SEQ ID NO: 109 - protein, 21 aa, Artificial Sequence
GSGEGRGSLLTCGDVEENPGP

SEQ ID NO: 110 - protein, 19 aa, Artificial Sequence
ATNFSLLKQAGDVEENPGP

SEQ ID NO: 111 - protein, 22 aa, Artificial Sequence
GSGATNFSLLKQAGDVEENPGP

SEQ ID NO: 112 - protein, 20 aa, Artificial Sequence
QCTNYALLKLAGDVESNPGP

SEQ ID NO: 113 - protein, 23 aa, Artificial Sequence
GSGQCTNYALLKLAGDVESNPGP

SEQ ID NO: 114 - protein, 22 aa, Artificial Sequence
VKQTLNFDLLKLAGDVESNPGP

SEQ ID NO: 115 - protein, 25 aa, Artificial Sequence
GSGVKQTLNFDLLKLAGDVESNPGP

SEQ ID NO: 116 - protein, 274 aa, Artificial Sequence
MLLLVTSLLLCELPHPAFLLIPQIVLTQSPAIMSASPGEKVTMTCSATSSVSYMHWYQQKSGTSPKRWIYDTSKLASGVPARFSGSGSGTSYSLTISSMEAEDAATYYCQQWSSNPLTFGAGTKLELKGGGGSGGGGSGGGSEVQLQQSGPELVKPGASVKMSCKASGYKFTSYVMHWVKQKPGQGLEWIGYINPYNDVTKYNEKFKGKATLTSDKSSSTAYMELSSLTSEDSAVHYCARGSYYDYDGFVYWGQGTLVTVSAESKYGPPCPPCP

SEQ ID NO: 117 - protein, 794 aa, Artificial Sequence
MLLLVTSLLLCELPHPAFLLIPQIVLTQSPAIMSASPGEKVTMTCSATSSVSYMHWYQQKSGTSPKRWIYDTSKLASGVPARFSGSGSGTSYSLTISSMEAEDAATYYCQQWSSNPLTFGAGTKLELKGGGGSGGGGSGGGSEVQLQQSGPELVKPGASVKMSCKASGYKFTSYVMHWVKQKPGQGLEWIGYINPYNDVTKYNEKFKGKATLTSDKSSSTAYMELSSLTSEDSAVHYCARGSYYDYDGFVYWGQGTLVTVSAESKYGPPCPPCPGGGGSCLENTGTFCSTALLITALALVCTLLYLKYKSRRSFIDEKKMPGSGATNFSLLKQAGDVEENPGPYGPGSMIHLGHILFLLLLPVAAAQTTPGERSSLPAFYPGTSGSCSGCGSLSLPLLAGLVAADAVASLLIVGAVFLCARPRRSPAQEDGKVYINMPGRGGGGSRVKFSRSADAPAYQQGQNQLYNELNLGRREEYDVLDKRRGRDPEMGGKPRRKNPQEGLYNELQKDKMAEAYSEIGMKGERRRGKGHDGLYQGLSTATKDTYDALHMQALPPRGSGEGRGSLLTCGDVEENPGPMGWIRGRRSRHSWEMSEFHNYNLDLKKSDFSTRWQKQRCPVVKSKCRENASPFFFCCFIAVAMGIRFIIMVTIWSAVFLNSLFNQEVQIPLTESYCGPCPKNWICYKNNCYQFFDESKNWYESQASCMSQNASLLKVYSKEDQDLLKLVKSYHWMGLVHIPTNGSWQWEDGSILSPNLLTIIEMQKGDCALYASSFKGYIENCSTPNTYICMQRTV

SEQ ID NO: 118 - DNA, 2382 bp, Artificial Sequence
atgctgctgctggtcacatctctgctgctgtgtgagctgccccatcccgcctttctgctgattccccagatcgtgctgacccagagccccgccatcatgtccgccagccccggcgagaaggtgaccatgacatgcagcgccaccagctccgtgtcctacatgcactggtaccagcagaagtccggcacctcccccaagaggtggatctacgacaccagcaagctggccagcggagtgcccgccagatttagcggcagcggaagcggaacatcctactctctgaccatcagcagcatggaggccgaggatgccgccacctattactgccagcagtggagcagcaaccctctgacctttggcgccggcaccaagctggaactgaaaggaggcggcggcagcggcggaggaggaagcggaggaggcagcgaggtgcagctccagcagtccggacccgagctggtcaagcccggagcttccgtcaagatgagctgcaaggccagcggctacaagttcaccagctacgtcatgcactgggtgaagcagaagcccggacaaggcctcgagtggatcggctatatcaacccctacaacgacgtgaccaagtacaacgagaagttcaagggcaaggccacactgacctccgacaagagctccagcacagcctacatggaactgagctctctgacaagcgaggattccgccgtgcactactgcgccagaggctcctactacgactacgacggctttgtgtactggggacaaggcacactggtcaccgtgagcgctgagagcaagtacggccccccttgccccccttgccccggcggaggcggaagctgtctggagaataccggaacattctgctccacagctctgctgattaccgctctggctctggtgtgcacactgctgtatctgaagtacaagtctagaaggagcttcatcgatgagaagaagatgcccggaagcggcgctaccaatttctctctgctgaaacaagccggagacgtcgaggagaaccccggcccctacggaccgggatccatgattcatctgggccacattctgtttctgctgctgctgcccgtggccgccgctcaaacaacccccggcgagagaagctctctgcccgctttctatcccggcacctccggcagctgttccggctgtggatctctgtccctccctctgctggctggactggtggctgccgatgctgtggcctctctgctgattgtgggagccgtgtttctgtgcgccagacccagaagaagccccgcccaagaagacggcaaggtgtacatcaacatgcccggcagaggcggaggaggcagcagagtcaagttctctagaagcgctgatgcccccgcttaccagcaaggccagaaccagctgtacaacgaactgaatctgggaagaagagaggagtacgatgtgctggacaagaggagaggaagagaccccgagatgggcggcaaacctaggaggaagaaccctcaagagggactgtacaacgagctgcagaaggataagatggccgaggcctactccgagatcggaatgaagggcgagagaagaagaggcaaaggacacgatggactgtaccaaggactgagcaccgccacaaaggacacatacgacgctctgcacatgcaagctctgcctcccagaggaagcggcgaaggaagaggctctctgctgacatgcggagatgtggaagagaatcccggccccatggggtggattcgtggtcggaggtctcgacacagctgggagatgagtgaatttcataattataacttggatctgaagaagagtgatttttcaacacgatggcaaaagcaaagatgtccagtagtcaaaagcaaatgtagagaaaatgcatctccattttttttctgctgcttcatcgctgtagccatgggaatccgtttcattattatggtaacaatatggagtgctgtattcctaaactcattattcaaccaagaagttcaaattcccttgaccgaaagttactgtggcccatgtcctaaaaactggatatgttacaaaaataactgctaccaattttttgatgagagtaaaaactggtatgagagccaggcttcttgtatgtctcaaaatgccagccttctgaaagtatacagcaaagaggaccaggatttacttaaactggtgaagtcatatcattggatgggactagtacacattccaacaaatggatcttggcagtgggaagatggctccattctctcacccaacctactaacaataattgaaatgcagaagggagactgtgcactctatgcctcgagctttaaaggctatatagaaaactgttcaactccaaatacgtacatctgcatgcaaaggactgtg

SEQ ID NO: 119 - protein, 10 aa, Artificial Sequence
DRHDSGLDSM

SEQ ID NO: 120 - protein, 7 aa, Artificial Sequence
ALAPYIP

SEQ ID NO: 121 - protein, 9 aa, Artificial Sequence
LDPETGEYL

SEQ ID NO: 122 - protein, 5 aa, Artificial Sequence
KFERQ

SEQ ID NO: 123 - protein, 14 aa, Artificial Sequence
KFERQKILDQRFFE

SEQ ID NO: 124 - protein, 5 aa, Artificial Sequence
QKILD

SEQ ID NO: 125 - protein, 5 aa, Artificial Sequence
QRDKV

SEQ ID NO: 126 - protein, 5 aa, Artificial Sequence
QRFFE

SEQ ID NO: 127 - protein, 5 aa, Artificial Sequence
QKKEL

SEQ ID NO: 128 - protein, 5 aa, Artificial Sequence
QFREL

SEQ ID NO: 129 - protein, 5 aa, Artificial Sequence
IKLDQ

SEQ ID NO: 130 - protein, 5 aa, Artificial Sequence
EFLKQ

SEQ ID NO: 131 - protein, 5 aa, Artificial Sequence
QKVFD

SEQ ID NO: 132 - protein, 5 aa, Artificial Sequence
QELLR

SEQ ID NO: 133 - protein, 5 aa, Artificial Sequence
QEFIK

SEQ ID NO: 134 - protein, 5 aa, Artificial Sequence
RKVEQ

SEQ ID NO: 135 - protein, 5 aa, Artificial Sequence
NRVVD

SEQ ID NO: 136 - protein, 5 aa, Artificial Sequence
NKKFE

SEQ ID NO: 137 - protein, 5 aa, Artificial Sequence
VKELQ

SEQ ID NO: 138 - protein, 5 aa, Artificial Sequence
VDKLN

SEQ ID NO: 139 - protein, 5 aa, Artificial Sequence
RIKEN

SEQ ID NO: 140 - protein, 5 aa, Artificial Sequence
DVVRQ

SEQ ID NO: 141 - protein, 5 aa, Artificial Sequence
QRIVE

SEQ ID NO: 142 - protein, 5 aa, Artificial Sequence
QLLRE

SEQ ID NO: 143 - protein, 5 aa, Artificial Sequence
IEKLQ

SEQ ID NO: 144 - protein, 5 aa, Artificial Sequence
QEKVF

SEQ ID NO: 145 - protein, 5 aa, Artificial Sequence
QDLKF

SEQ ID NO: 146 - protein, 5 aa, Artificial Sequence
VKKDQ

SEQ ID NO: 147 - protein, 22 aa, Artificial Sequence
DRHDSGLDSMGSGSGALAPYIP

SEQ ID NO: 148 - protein, 30 aa, Artificial Sequence
MDSKGSSQKGSRLLLLLVVSNLLLPQGVVG

SEQ ID NO: 149 - protein, 18 aa, Artificial Sequence
MDWTWILFLVAAATRVHS

SEQ ID NO: 150 - protein, 20 aa, Artificial Sequence
METPAQLLFLLLLWLPDTTG

SEQ ID NO: 151 - protein, 22 aa, Artificial Sequence
MLGSNSGQRVVFTILLVAPAYS

SEQ ID NO: 152 - protein, 17 aa, Artificial Sequence
MKCLLYLAFLFIGVNCA

SEQ ID NO: 153 - protein, 15 aa, Artificial Sequence
MWLVSLAIVTACAGA

SEQ ID NO: 154 - protein, 15 aa, Artificial Sequence
MFVFLVLLPLVSSQC

SEQ ID NO: 155 - protein, 36 aa, Artificial Sequence
CKICMDRNIAIVFVPCGHLVTCKQCAEAVDKCPMCY

SEQ ID NO: 156 - protein, 36 aa, Artificial Sequence
CKVCMDKEVSVVFIPCGHLVVCQECAPSLRKCPICR

SEQ ID NO: 157 - protein, 36 aa, Artificial Sequence; identical to SEQ ID NO: 156

SEQ ID NO: 158 - protein, 35 aa, Artificial Sequence
CKVCLDRAVSIVFVPCGHLVCAECAPGLQLCPICR

SEQ ID NO: 159 - protein, 36 aa, Artificial Sequence
CKICMDRHIAVVFIPCGHLVTCKQCAEAVDRCPMCS

SEQ ID NO: 160 - DNA, 2106 bp, Artificial Sequence
atgctgctgctggtgacaagcctgctgctgtgcgagctgccccaccccgccttcctgctgatccctcagatcgtgctgacacagagccccgccatcatgagcgcctctcccggcgaaaaggtgaccatgacctgcagcgccacaagcagcgtgagctacatgcactggtatcagcagaagagcggcacaagcccgaagagatggatctacgacacaagcaagctggcaagcggcgtgcccgctagattcagcggcagcggcagcggcactagctacagcctgaccatcagcagcatggaggccgaggacgccgccacctactactgtcagcagtggagcagcaaccccctgaccttcggggccggcaccaaactggagctaaagggcggaggcggcagcggaggcggggggagtggtggtgggtctgaagtacaactgcagcaaagcggccccgagctggtgaagcccggcgcaagcgtgaagatgagctgcaaggcaagcggctacaagttcacaagctacgtgatgcactgggtgaagcagaagcccggccaaggcctggagtggatcggctacatcaacccctacaacgacgtgaccaagtacaacgagaagttcaagggcaaggccaccctgactagcgataagagcagcagcaccgcctacatggagctgagcagcctgacaagcgaagacagcgccgtgcactactgcgctagaggcagctactacgactacgacggcttcgtgtactggggccaaggcaccttagtaaccgtgagcgctgagagcaagtacggaccgccctgccccccctgccccggcgggggcggctcctgcctggagaacaccggcaccttctgcagcaccgccctgctgatcaccgccctggccctggtgtgcaccctgctgtacctgaagtacaagagcagaagaagcttcatcgacgagaagaagatgcccggcagcggcgccacaaacttcagcctgctgaagcaagccggcgacgtggaggagaaccccggccccggatccatgcttctcctggtgacaagccttctgctctgtgagttaccacacccagcattcctcctgatcccacgcaaagtgtgtaacggaataggtattggtgaatttaaagactcactctccataaatgctacgaatattaaacacttcaaaaactgcacctccatcagtggcgatctccacatcctgccggtggcatttaggggtgactccttcacacatactcctcctctggacccacaggaactggatattctgaaaaccgtaaaggaaatcacagggtttttgctgattcaggcttggcctgaaaacaggacggacctccatgcctttgagaacctagaaatcatacgcggcaggaccaagcaacatggtcagttttctcttgcagtcgtcagcctgaacataacatccttgggattacgctccctcaaggagataagtgatggagatgtgataatttcaggaaacaaaaatttgtgctatgcaaatacaataaactggaaaaaactgtttgggacctccggtcagaaaaccaaaattataagcaacagaggtgaaaacagctgcaaggccacaggccaggtctgccatgccttgtgctcccccgagggctgctggggcccggagcccagggactgcgtctcttgccggaatgtcagccgaggcagggaatgcgtggacaagtgcaaccttctggagggtgagccaagggagtttgtggagaactctgagtgcatacagtgccacccagagtgcctgcctcaggccatgaacatcacctgcacaggacggggaccagacaactgtatccagtgtgcccactacattgacggcccccactgcgtcaagacctgcccggcaggagtcatgggagaaaacaacaccctggtctggaagtacgcagacgccggccatgtgtgccacctgtgccatccaaactgcacctacggatgcactgggccaggtcttgaaggctgtccaacgaatgggcctaagatcccgtccatcgccactgggatggtgggggccctcctcttgctgctggtggtggccctggggatcggcctcttcatg

SEQ ID NO: 161 - protein, 702 aa, Artificial Sequence
MLLLVTSLLLCELPHPAFLLIPQIVLTQSPAIMSASPGEKVTMTCSATSSVSYMHWYQQKSGTSPKRWIYDTSKLASGVPARFSGSGSGTSYSLTISSMEAEDAATYYCQQWSSNPLTFGAGTKLELKGGGGSGGGGSGGGSEVQLQQSGPELVKPGASVKMSCKASGYKFTSYVMHWVKQKPGQGLEWIGYINPYNDVTKYNEKFKGKATLTSDKSSSTAYMELSSLTSEDSAVHYCARGSYYDYDGFVYWGQGTLVTVSAESKYGPPCPPCPGGGGSCLENTGTFCSTALLITALALVCTLLYLKYKSRRSFIDEKKMPGSGATNFSLLKQAGDVEENPGPGSMLLLVTSLLLCELPHPAFLLIPRKVCNGIGIGEFKDSLSINATNIKHFKNCTSISGDLHILPVAFRGDSFTHTPPLDPQELDILKTVKEITGFLLIQAWPENRTDLHAFENLEIIRGRTKQHGQFSLAVVSLNITSLGLRSLKEISDGDVIISGNKNLCYANTINWKKLFGTSGQKTKIISNRGENSCKATGQVCHALCSPEGCWGPEPRDCVSCRNVSRGRECVDKCNLLEGEPREFVENSECIQCHPECLPQAMNITCTGRGPDNCIQCAHYIDGPHCVKTCPAGVMGENNTLVWKYADAGHVCHLCHPNCTYGCTGPGLEGCPTNGPKIPSIATGMVGALLLLLVVALGIGLFM

SEQ ID NO: 162 - DNA, 2187 bp, Artificial Sequence
atgctgctgctggtgacaagcctgctgctgtgcgagctgccccaccccgccttcctgctgatccctcagatcgtgctgacacagagccccgccatcatgagcgcctctcccggcgaaaaggtgaccatgacctgcagcgccacaagcagcgtgagctacatgcactggtatcagcagaagagcggcacaagcccgaagagatggatctacgacacaagcaagctggcaagcggcgtgcccgctagattcagcggcagcggcagcggcactagctacagcctgaccatcagcagcatggaggccgaggacgccgccacctactactgtcagcagtggagcagcaaccccctgaccttcggggccggcaccaaactggagctaaagggcggaggcggcagcggaggcggggggagtggtggtgggtctgaagtacaactgcagcaaagcggccccgagctggtgaagcccggcgcaagcgtgaagatgagctgcaaggcaagcggctacaagttcacaagctacgtgatgcactgggtgaagcagaagcccggccaaggcctggagtggatcggctacatcaacccctacaacgacgtgaccaagtacaacgagaagttcaagggcaaggccaccctgactagcgataagagcagcagcaccgcctacatggagctgagcagcctgacaagcgaagacagcgccgtgcactactgcgctagaggcagctactacgactacgacggcttcgtgtactggggccaaggcaccttagtaaccgtgagcgctgagagcaagtacggaccgccctgccccccctgccccggcgggggcggctcctgcctggagaacaccggcaccttctgcagcaccgccctgctgatcaccgccctggccctggtgtgcaccctgctgtacctgaagtacaagagcagaagaagcttcatcgacgagaagaagatgcccgggggcgggggctccgacagacatgatagcggcctggacagcatgggcagcggcagcggggccctggccccctacatccccggcagcggcgccacaaacttcagcctgctgaagcaagccggcgacgtggaggagaaccccggccccggatccatgcttctcctggtgacaagccttctgctctgtgagttaccacacccagcattcctcctgatcccacgcaaagtgtgtaacggaataggtattggtgaatttaaagactcactctccataaatgctacgaatattaaacacttcaaaaactgcacctccatcagtggcgatctccacatcctgccggtggcatttaggggtgactccttcacacatactcctcctctggacccacaggaactggatattctgaaaaccgtaaaggaaatcacagggtttttgctgattcaggcttggcctgaaaacaggacggacctccatgcctttgagaacctagaaatcatacgcggcaggaccaagcaacatggtcagttttctcttgcagtcgtcagcctgaacataacatccttgggattacgctccctcaaggagataagtgatggagatgtgataatttcaggaaacaaaaatttgtgctatgcaaatacaataaactggaaaaaactgtttgggacctccggtcagaaaaccaaaattataagcaacagaggtgaaaacagctgcaaggccacaggccaggtctgccatgccttgtgctcccccgagggctgctggggcccggagcccagggactgcgtctcttgccggaatgtcagccgaggcagggaatgcgtggacaagtgcaaccttctggagggtgagccaagggagtttgtggagaactctgagtgcatacagtgccacccagagtgcctgcctcaggccatgaacatcacctgcacaggacggggaccagacaactgtatccagtgtgcccactacattgacggcccccactgcgtcaagacctgcccggcaggagtcatgggagaaaacaacaccctggtctggaagtacgcagacgccggccatgtgtgccacctgtgccatccaaactgcacctacggatgcactgggccaggtcttgaaggctgtccaacgaatgggcctaagatcccgtccatcgccactgggatggtgggggccctcctcttgctgctggtggtggccctggggatcggcctcttcatg

SEQ ID NO: 163 - protein, 729 aa, Artificial Sequence
MLLLVTSLLLCELPHPAFLLIPQIVLTQSPAIMSASPGEKVTMTCSATSSVSYMHWYQQKSGTSPKRWIYDTSKLASGVPARFSGSGSGTSYSLTISSMEAEDAATYYCQQWSSNPLTFGAGTKLELKGGGGSGGGGSGGGSEVQLQQSGPELVKPGASVKMSCKASGYKFTSYVMHWVKQKPGQGLEWIGYINPYNDVTKYNEKFKGKATLTSDKSSSTAYMELSSLTSEDSAVHYCARGSYYDYDGFVYWGQGTLVTVSAESKYGPPCPPCPGGGGSCLENTGTFCSTALLITALALVCTLLYLKYKSRRSFIDEKKMPGGGGSDRHDSGLDSMGSGSGALAPYIPGSGATNFSLLKQAGDVEENPGPGSMLLLVTSLLLCELPHPAFLLIPRKVCNGIGIGEFKDSLSINATNIKHFKNCTSISGDLHILPVAFRGDSFTHTPPLDPQELDILKTVKEITGFLLIQAWPENRTDLHAFENLEIIRGRTKQHGQFSLAVVSLNITSLGLRSLKEISDGDVIISGNKNLCYANTINWKKLFGTSGQKTKIISNRGENSCKATGQVCHALCSPEGCWGPEPRDCVSCRNVSRGRECVDKCNLLEGEPREFVENSECIQCHPECLPQAMNITCTGRGPDNCIQCAHYIDGPHCVKTCPAGVMGENNTLVWKYADAGHVCHLCHPNCTYGCTGPGLEGCPTNGPKIPSIATGMVGALLLLLVVALGIGLFM

SEQ ID NO: 164 - DNA, 558 bp, Artificial Sequence
atgagatacatgattctgggactgctggctctggctgctgtgtgtagcgccgccaaaaaggtggaattcaaggagcccgcttgcaacgtgacctttaagtccgaggccaacgagtgcaccacactgatcaagtgcaccaccgagcacgagaagctgatcattagacacaaggacaagatcggaagatacgccgtgtacgccatctggcagcccggcgacaccaacgactacaacgtcaccgtgttccaaggcgagaatagaaagaccttcatgtataagttccccttctacgagatgtgcgacatcaccatgtacatgagcaagcagtacaagctgtggccccctcagaagtgtctggagaacaccggcaccttctgtagcacagctctgctgatcacagctctggctctggtgtgcacactgctctatctgaagtacaagtctagaaggagcttcatcgacgagaagaagatgcccgggggcgggggctccgacagacatgatagcggcctggacagcatgggcagcggcagcggggccctggccccctacatcccc

SEQ ID NO: 165 - protein, 186 aa, Artificial Sequence
MRYMILGLLALAAVCSAAKKVEFKEPACNVTFKSEANECTTLIKCTTEHEKLIIRHKDKIGKYAVYAIWQPGDTNDYNVTVFQGENRKTFMYKFPFYEMCDITMYMSKQYKLWPPQKCLENTGTFCSTALLITALALVCTLLYLKYKSRRSFIDEKKMPGGGGSDRHDSGLDSMGSGSGALAPYIP

SEQ ID NO: 166 - DNA, 1959 bp, Artificial Sequence
atgattcatctgggccacattctgtttctgctgctgctgcccgtggccgccgctcaaacaacccccggcgagagaagctctctgcccgctttctatcccggcacctccggcagctgttccggctgtggatctctgtccctccctctgctggctggactggtggctgccgatgctgtggcctctctgctgattgtgggagccgtgtttctgtgcgccagacccagaagaagccccgcccaagacggcaaggtgtacatcaacatgcccggcagaggcggaggaggcagcagagtcaagttctctagaagcgctgatgcccccgcttaccagcaaggccagaaccagctgtacaacgaactgaatctgggaagaagagaggagtacgatgtgctggacaagaggagaggaagagaccccgagatgggcggcaaacctaggaggaagaaccctcaagagggactgtacaacgagctgcagaaggataagatggccgaggcctactccgagatcggaatgaagggcgagagaagaagaggcaaaggacacgatggactgtaccaaggactgagcaccgccacaaaggacacatacgacgctctgcacatgcaagctctgcctcccagaggaagcggcgaaggaagaggctctctgctgacatgcggagatgtggaagagaatcccggccccatggggtggattcgtggtcggaggtctcgacacagctgggagatgagtgaatttcataattataacttggatctgaagaagagtgatttttcaacacgatggcaaaagcaaagatgtccagtagtcaaaagcaaatgtagagaaaatgcatctccattttttttctgctgcttcatcgctgtagccatgggaatccgtttcattattatggtaacaatatggagtgctgtattcctaaactcattattcaaccaagaagttcaaattcccttgaccgaaagttactgtggcccatgtcctaaaaactggatatgttacaaaaataactgctaccaattttttgatgagagtaaaaactggtatgagagccaggcttcttgtatgtctcaaaatgccagccttctgaaagtatacagcaaagaggaccaggatttacttaaactggtgaagtcatatcattggatgggactagtacacattccaacaaatggatcttggcagtgggaagatggctccattctctcacccaacctactaacaataattgaaatgcagaagggagactgtgcactctatgcctcgagctttaaaggctatatagaaaactgttcaactccaaatacgtacatctgcatgcaaaggactgtgggcagcggcgccacaaatttctctctgctgaagcaagccggcgacgtggaggagaatcccggacccatgagatacatgattctgggactgctggctctggctgctgtgtgtagcgccgccaaaaaggtggaattcaaggagcccgcttgcaacgtgacctttaagtccgaggccaacgagtgcaccacactgatcaagtgcaccaccgagcacgagaagctgatcattagacacaaggacaagatcggaagatacgccgtgtacgccatctggcagcccggcgacaccaacgactacaacgtcaccgtgttccaaggcgagaatagaaagaccttcatgtataagttccccttctacgagatgtgcgacatcaccatgtacatgagcaagcagtacaagctgtggccccctcagaagtgtctggagaacaccggcaccttctgtagcacagctctgctgatcacagctctggctctggtgtgcacactgctctatctgaagtacaagtctagaaggagcttcatcgacgagaagaagatgcccgggggcgggggctccgacagacatgatagcggcctggacagcatgggcagcggcagcggggccctggccccctacatcccc

SEQ ID NO: 167 - protein, 653 aa, Artificial Sequence
MIHLGHILFLLLLPVAAAQTTPGERSSLPAFYPGTSGSCSGCGSLSLPLLAGLVAADAVASLLIVGAVFLCARPRRSPAQDGKVYINMPGRGGGGSRVKFSRSADAPAYQQGQNQLYNELNLGRREEYDVLDKRRGRDPEMGGKPRRKNPQEGLYNELQKDKMAEAYSEIGMKGERRRGKGHDGLYQGLSTATKDTYDALHMQALPPRGSGEGRGSLLTCGDVEENPGPMGWIRGRRSRHSWEMSEFHNYNLDLKKSDFSTRWQKQRCPVVKSKCRENASPFFFCCFIAVAMGIRFIIMVTIWSAVFLNSLFNQEVQIPLTESYCGPCPKNWICYKNNCYQFFDESKNWYESQASCMSQNASLLKVYSKEDQDLLKLVKSYHWMGLVHIPTNGSWQWEDGSILSPNLLTIIEMQKGDCALYASSFKGYIENCSTPNTYICMQRTVGSGATNFSLLKQAGDVEENPGPMRYMILGLLALAAVCSAAKKVEFKEPACNVTFKSEANECTTLIKCTTEHEKLIIRHKDKIGKYAVYAIWQPGDTNDYNVTVFQGENRKTFMYKFPFYEMCDITMYMSKQYKLWPPQKCLENTGTFCSTALLITALALVCTLLYLKYKSRRSFIDEKKMPGGGGSDRHDSGLDSMGSGSGALAPYIP

SEQ ID NO: 168 - DNA, 1335 bp, Artificial Sequence
atgattcatctgggccacattctgtttctgctgctgctgcccgtggccgccgctcaaacaacccccggcgagagaagctctctgcccgctttctatcccggcacctccggcagctgttccggctgtggatctctgtccctccctctgctggctggactggtggctgccgatgctgtggcctctctgctgattgtgggagccgtgtttctgtgcgccagacccagaagaagccccgcccaagacggcaaggtgtacatcaacatgcccggcagaggcggaggaggcagcagagtcaagttctctagaagcgctgatgcccccgcttaccagcaaggccagaaccagctgtacaacgaactgaatctgggaagaagagaggagtacgatgtgctggacaagaggagaggaagagaccccgagatgggcggcaaacctaggaggaagaaccctcaagagggactgtacaacgagctgcagaaggataagatggccgaggcctactccgagatcggaatgaagggcgagagaagaagaggcaaaggacacgatggactgtaccaaggactgagcaccgccacaaaggacacatacgacgctctgcacatgcaagctctgcctcccagaggaagcggcgaaggaagaggctctctgctgacatgcggagatgtggaagagaatcccggccccatggggtggattcgtggtcggaggtctcgacacagctgggagatgagtgaatttcataattataacttggatctgaagaagagtgatttttcaacacgatggcaaaagcaaagatgtccagtagtcaaaagcaaatgtagagaaaatgcatctccattttttttctgctgcttcatcgctgtagccatgggaatccgtttcattattatggtaacaatatggagtgctgtattcctaaactcattattcaaccaagaagttcaaattcccttgaccgaaagttactgtggcccatgtcctaaaaactggatatgttacaaaaataactgctaccaattttttgatgagagtaaaaactggtatgagagccaggcttcttgtatgtctcaaaatgccagccttctgaaagtatacagcaaagaggaccaggatttacttaaactggtgaagtcatatcattggatgggactagtacacattccaacaaatggatcttggcagtgggaagatggctccattctctcacccaacctactaacaataattgaaatgcagaagggagactgtgcactctatgcctcgagctttaaaggctatatagaaaactgttcaactccaaatacgtacatctgcatgcaaaggactgtg

SEQ ID NO: 169 - protein, 445 aa, Artificial Sequence
MIHLGHILFLLLLPVAAAQTTPGERSSLPAFYPGTSGSCSGCGSLSLPLLAGLVAADAVASLLIVGAVFLCARPRRSPAQDGKVYINMPGRGGGGSRVKFSRSADAPAYQQGQNQLYNELNLGRREEYDVLDKRRGRDPEMGGKPRRKNPQEGLYNELQKDKMAEAYSEIGMKGERRRGKGHDGLYQGLSTATKDTYDALHMQALPPRGSGEGRGSLLTCGDVEENPGPMGWIRGRRSRHSWEMSEFHNYNLDLKKSDFSTRWQKQRCPVVKSKCRENASPFFFCCFIAVAMGIRFIIMVTIWSAVFLNSLFNQEVQIPLTESYCGPCPKNWICYKNNCYQFFDESKNWYESQASCMSQNASLLKVYSKEDQDLLKLVKSYHWMGLVHIPTNGSWQWEDGSILSPNLLTIIEMQKGDCALYASSFKGYIENCSTPNTYICMQRTV

SEQ ID NO: 170 - DNA, 1044 bp, Artificial Sequence
atgctgctgctcgtgaccagcctgctgctgtgcgaactgccccaccctgcctttctgctgatccccgacatcgtgatgacccagagccctagcagcctggccgtgtccgtgggcgagaaagtgaccatgagctgcaagagcagccagagcctgctgttcagcagcaaccagaagaactacctggcctggtatcagcagaagcccggccagagccccaagctgctgatctactgggccagcaccagagaaagcggcgtgcccgatagattcaccggctctggcagcggcaccgacttcaccctgacaatcagcagcgtgaaggccgaggacctggctgtgtactactgccagcagttctacagcttcccccggacctttggcggaggcaccaagctggaaatcaagagaggcggcggaggaagcggaggcggaggatctggcggagggggctccggagggggaggctctgaagtgcagctggtggaaagtggcggcggactcgtgaagcctggcggctctctgaagctgagctgtgccgccagcggcttcaccttcagcagctacgccatgtcctgggtgcgccagacccccgagaagagactggaatgggtggccacagtgtcctacggcggcagctacaccttctaccccgacaatgtgaagggccggttcaccatcagccgggacaacgccaagaacaacctgtacctgcagatgagccacctgaagtccgaggataccgccatgtactattgcgccagagactacgactacgatttcttcgacagctggggccagggcaccaccgtgacagtgtccagcgagtctaagtacggaccgccctgccccccctgccccggcgggggcggcagctgcctggagaacaccggcaccttctgcagcaccgccctgctgatcaccgccctggccctggtgtgcaccctgctgtacctgaagtacaagagcagaagaagcttcatcgacgagaagaagatgcccggcgggggcggcagcgacagacacgacagcggcctggacagcatg

SEQ ID NO: 171 - protein, 348 aa, Artificial Sequence
MLLLVTSLLLCELPHPAFLLIPDIVMTQSPSSLAVSVGEKVTMSCKSSQSLLFSSNQKNYLAWYQQKPGQSPKLLIYWASTRESGVPDRFTGSGSGTDFTLTISSVKAEDLAVYYCQQFYSFPRTFGGGTKLEIKRGGGGSGGGGSGGGGSGGGGSEVQLVESGGGLVKPGGSLKLSCAASGFTFSSYAMSWVRQTPEKRLEWVATVSYGGSYTFYPDNVKGRFTISRDNAKNNLYLQMSHLKSEDTAMYYCARDYDYDFFDSWGQGTTVTVSSESKYGPPCPPCPGGGGSCLENTGTFCSTALLITALALVCTLLYLKYKSRRSFIDEKKMPGGGGSDRHDSGLDSM

SEQ ID NO: 172 - protein, 12 aa, Artificial Sequence
ESKYGPPCPPCP

SEQ ID NO: 173 - protein, 10 aa, Artificial Sequence
GGGGSGGGGS

SEQ ID NO: 174 - protein, 17 aa, Artificial Sequence
VTVDCNLSMMWMRFFVC

SEQ ID NO: 175 - protein, 21 aa, Artificial Sequence
TLLVYLFSLVVLVLLTVGVSA

SEQ ID NO: 176 - protein, 5 aa, Artificial Sequence
RLRFI

SEQ ID NO: 177 - protein, 21 aa, Artificial Sequence
YTLMMVAVIQVFWGLYVKGWL

SEQ ID NO: 178 - protein, 12 aa, Artificial Sequence
HRHFPWMFSDQW